European Patent Application EP 4 628 591 A1, published October 8, 2025. Title: Method for producing CaAIBZ1 gene editing chili pepper to enhance drought tolerance. Applicant: TOOLGEN INCORPORATED. Application KR. The sequence listing filed with the application follows.

SEQUENCE LISTING (6 sequences)

SEQ ID NO: 1 - DNA, 23 bp, synthetic construct
  source 1..23: mol_type = other DNA
atcattgttgccgatgtactcgg

SEQ ID NO: 2 - DNA, 23 bp, synthetic construct
  source 1..23: mol_type = other DNA
ctcagttcgttgcctcaagaagg

SEQ ID NO: 3 - DNA, 23 bp, synthetic construct
  source 1..23: mol_type = other DNA
cactacatcaaattggcatgtgg

SEQ ID NO: 4 - DNA, 23 bp, synthetic construct
  source 1..23: mol_type = other DNA
tgccgatgtactcgggcaactgg

SEQ ID NO: 5 - DNA, 20 bp, synthetic construct
  source 1..20: mol_type = other DNA
ttcgataagaaccttccaaa

SEQ ID NO: 6 - DNA, 20 bp, synthetic construct
  source 1..20: mol_type = other DNA
ttgagcctttcttcaatcat